European Patent Application EP 4 176 898 A1, published May 10, 2023. Title: Pan Sars-CoV2 Vaccine Antigen. Applicant: Charite. The sequence listing filed with the application follows.

SEQUENCE LISTING (60 sequences)

SEQ ID NO: 1 - protein, 1128 aa, Artificial Sequence
  PanCoVac
MDWTWILFLVAAATRVHSRPDTRYVLAATPKYKFVRIAAFLLPSLATVAAKLWAQCVQLAATEAFEKMVSLAAALWEIQQVVAACTDDNALAYYAAVTDTPKGPKAATEVPANSTVLAADLKGKYVQIAALSFKELLVYAAIPRRNVATLAAMMISAGFSLRGRKRRSMFIFLLFLTAAKGIYQTSNFRVAAVRFPNITNLCPFGEVFNATRFASVYAWNRKRSNCVADYSVLYNSAAGYQPYRVVVLSFELLAACVNFNFNGLTGTGVLTAANLLLQYGSFCTQLNRALAASFIEDLLFNKVTLADAGFAAARDLICAQKFNGLTVLPPLLAAGWTFGAGAALQIPFAMQMAYRFNGIGVTQNVLYENQKAAALGKLQDVVNQNAQALNTLVKQLSSNFGAISSVLNDILSRLDKVEAEVQIDRLITGRLQSLQTYVTQQLIRAAEIRASANLAATKMSECVLGQSKRVDFCGKGYHLMSAAAPHGVVFLHVTYVAAQIITTDNTFVSGNCDVVIGIAANTVYDPLQPELDSFKEELDKYFKNHTSPDVDLGDISGINASVVNIQKEIDRLNEVAKNLNESLIDLQELGKYEQYIKWPWYIAAWLGFIAGLIAIVMVTIAACCKFDEDDSEPVLKGVKLHYRGRKRRSMYSFVSEETGTLIVNSVLLFLAFVVFLLVTLAILTALRLCAYCCNIVNVSLVKAAYVYSRVKNLRGRKRRSNRNRFLYIIKLAAFLWLLWPVTLACFVLAAVYRINWAAASFRLFARTRSMWSFNPETNILLNVPLAAESELVIGAVIAAGRCDIKDLPKEITVATSRTLSYYKLGASQRVAGDAARYRIGNYKLNTRGRKRRSKQRRPQGLPNNTASWFTALTQHGKEAAFPRGQGVPINAALSPRWYFYYLGTGPEAAAVLQLPQGTTLPKGFYAEGSRGGSQASSRSSSRSRAAALALLLLDRLNQLESKAAKGQQQQGQTVTKKSAAEASKKPRQKRTATKAAYNVTQAFGRRGPEQTQGNFAALIRQGTDYKHWPQIAQFAPSASAFFGMSRIGMEVTPSGTWLTYAAVILLNKHIDAYKTFPPTEPKKDKKKKADETRGRKRRSTYEGNSPFHPLADNKFALAARARSVSPKL

SEQ ID NO: 2 - protein, 1110 aa, Artificial Sequence
  PanCoVac without leader sequence
RPDTRYVLAATPKYKFVRIAAFLLPSLATVAAKLWAQCVQLAATEAFEKMVSLAAALWEIQQVVAACTDDNALAYYAAVTDTPKGPKAATEVPANSTVLAADLKGKYVQIAALSFKELLVYAAIPRRNVATLAAMMISAGFSLRGRKRRSMFIFLLFLTAAKGIYQTSNFRVAAVRFPNITNLCPFGEVFNATRFASVYAWNRKRSNCVADYSVLYNSAAGYQPYRVVVLSFELLAACVNFNFNGLTGTGVLTAANLLLQYGSFCTQLNRALAASFIEDLLFNKVTLADAGFAAARDLICAQKFNGLTVLPPLLAAGWTFGAGAALQIPFAMQMAYRFNGIGVTQNVLYENQKAAALGKLQDVVNQNAQALNTLVKQLSSNFGAISSVLNDILSRLDKVEAEVQIDRLITGRLQSLQTYVTQQLIRAAEIRASANLAATKMSECVLGQSKRVDFCGKGYHLMSAAAPHGVVFLHVTYVAAQIITTDNTFVSGNCDVVIGIAANTVYDPLQPELDSFKEELDKYFKNHTSPDVDLGDISGINASVVNIQKEIDRLNEVAKNLNESLIDLQELGKYEQYIKWPWYIAAWLGFIAGLIAIVMVTIAACCKFDEDDSEPVLKGVKLHYRGRKRRSMYSFVSEETGTLIVNSVLLFLAFVVFLLVTLAILTALRLCAYCCNIVNVSLVKAAYVYSRVKNLRGRKRRSNRNRFLYIIKLAAFLWLLWPVTLACFVLAAVYRINWAAASFRLFARTRSMWSFNPETNILLNVPLAAESELVIGAVIAAGRCDIKDLPKEITVATSRTLSYYKLGASQRVAGDAARYRIGNYKLNTRGRKRRSKQRRPQGLPNNTASWFTALTQHGKEAAFPRGQGVPINAALSPRWYFYYLGTGPEAAAVLQLPQGTTLPKGFYAEGSRGGSQASSRSSSRSRAAALALLLLDRLNQLESKAAKGQQQQGQTVTKKSAAEASKKPRQKRTATKAAYNVTQAFGRRGPEQTQGNFAALIRQGTDYKHWPQIAQFAPSASAFFGMSRIGMEVTPSGTWLTYAAVILLNKHIDAYKTFPPTEPKKDKKKKADETRGRKRRSTYEGNSPFHPLADNKFALAARARSVSPKL

SEQ ID NO: 3 - DNA, 3387 bp, Artificial Sequence
  PanCoVac
atggactggacctggatcctgtttctggtggccgctgccacaagagtgcactcaagacccgataccagatacgtgctggccgccacacctaagtacaagttcgtccggatcgccgccttcctgctgccttctttggctacagtggccgccaaactgtgggcccagtgtgttcaactggccgctacagaggccttcgagaagatggtgtctctggctgccgctctgtgggagatccagcaagtggtggctgcctgcaccgacgataatgccctggcctattatgccgccgtgacagacacaccaaagggccctaaagccgccacagaggtgccagccaattctacagtgctggcagccgacctgaagggcaaatacgtgcagatcgccgctctgagcttcaaagaactgctggtgtacgccgccattcctcggagaaatgtggctaccctggctgccatgatgatcagcgccggctttagcctgagaggccggaagcggagatccatgtttatctttctgctgttcctgaccgccgccaagggcatctaccagaccagcaatttcagagtggctgccgtgcggttccccaacatcaccaatctgtgccctttcggcgaggtgttcaatgccacaagatttgccagcgtgtacgcctggaaccggaagagaagcaactgcgtggccgactacagcgtgctgtacaatagcgccgctggctaccagccttacagagtggtggtgctgagcttcgagctgctggctgcttgcgtgaacttcaacttcaacggcctgaccggcaccggcgttctgacagctgctaatctgctgctgcagtacggcagcttctgcacccagctgaatagagccctggccgccagcttcatcgaggacctgctgttcaacaaagtgaccctggccgatgccggatttgccgctgctagggatctgatctgcgcccagaagtttaacggactgaccgtgctgcctcctctgcttgctgccggatggacatttggagctggtgctgccctgcagatccccttcgctatgcagatggcctaccggttcaatggcatcggcgtgacccagaatgtgctgtacgagaaccagaaggccgctgctctgggcaagctgcaggatgtggtcaaccagaatgcccaggctctgaacaccctggtcaagcagctgagcagcaacttcggcgccatcagctccgtgctgaacgacatcctgagccggctggataaggtggaagccgaggtgcagattgaccggctgatcacaggcagactgcagagcctgcagacctacgtgacacagcagctgatcagggccgctgagattagagcctctgccaacctggccgcaacaaagatgagcgagtgtgtgctgggccagagcaagagagtggacttttgcggcaagggctaccacctgatgtcagctgctgctcctcacggcgtggtgtttctgcacgtgacatatgtggccgctcagatcatcaccaccgacaacaccttcgtgtccggcaactgcgacgtggtcattggaatcgccgccaataccgtgtacgaccctctgcagcctgagctggactccttcaaagaggaactggacaagtacttcaagaaccacacaagccccgacgtggacctgggcgatatctctggcatcaatgccagcgtcgtgaacatccagaaagagatcgacagactgaacgaggtggccaagaacctgaacgagagcctgatcgacctgcaagagctggggaagtacgagcagtacatcaagtggccctggtacattgccgcctggctgggctttatcgccggactgattgccatcgtgatggtcacaatcgccgcttgctgcaagttcgacgaggacgatagcgagcctgtgctgaagggcgtgaagctgcactacagaggacgcaagaggcggagcatgtacagctttgtgtccgaggaaaccggcacactgatcgtgaatagcgtgctcctgttcctggccttcgtcgtgttcctgctggtcacactggccatcctgacagccctgagactgtgcgcctactgctgcaacatcgtgaacgtgtccctggttaaggccgcctacgtgtacagcagagtgaagaacctgagaggacgcaagaggcggagcaacagaaacagattcctgtacattatcaagctggctgccttcctgtggttgctgtggcctgtgacactggcctgttttgttctggccgccgtgtaccggatcaattgggctgccgcctccttccggctgtttgccagaaccagatctatgtggtccttcaatcccgagacaaacatcctgctgaatgtgcccctggcagctgagagcgagctggttattggagccgtgatcgctgccggaagatgcgacatcaaggatctgcccaaagaaatcaccgtggccaccagcagaaccctgagctactataagctgggcgcctctcagagagtggcaggcgacgctgccagatacagaatcggcaactacaagctgaacaccagaggcagaaaaaggcggtccaaacagagaaggcctcagggcctgcctaacaacaccgccagctggtttactgccctgactcagcacggcaaagaagccgcctttcctagaggacagggcgtgccaatcaacgccgcactgagccctagatggtacttctactacctcggcacaggcccagaggctgcagctgttctgcaactgcctcagggaaccacactgcctaagggcttttacgccgagggctctagaggcggaagccaggcctctagcagaagcagctctagaagcagagccgctgcactggcattgctgctgctggacaggctgaatcagctggaaagcaaggccgctaagggccagcagcaacagggacagaccgtgaccaagaagtctgccgccgaggccagcaagaagcccagacagaaaagaaccgccaccaaagccgcctacaatgtgacccaggccttcggcagaagaggccctgaacagacccagggcaatttcgctgccctgattagacagggcaccgactacaagcactggccccagattgcccagtttgcccctagcgcctctgcctttttcggcatgtctcggatcggcatggaagtgacccctagcggcacatggctgacatacgccgctgtgattctgctgaacaagcacatcgacgcctacaagacattccctccaaccgagcctaagaaggacaagaagaagaaggccgacgagacacgcggaagaaagcggagaagcacctacgagggcaacagcccttttcaccctctggccgataacaagttcgccctcgctgctagagccagaagcgtgtcacctaaactgtaa

SEQ ID NO: 4 - protein, 143 aa, Artificial Sequence
  first nonstructural protein epitope polypeptide sequence
RPDTRYVLAATPKYKFVRIAAFLLPSLATVAAKLWAQCVQLAATEAFEKMVSLAAALWEIQQVVAACTDDNALAYYAAVTDTPKGPKAATEVPANSTVLAADLKGKYVQIAALSFKELLVYAAIPRRNVATLAAMMISAGFSL

SEQ ID NO: 5 - protein, 29 aa, Artificial Sequence
  Accessory protein epitope polypeptide sequence
TYEGNSPFHPLADNKFALAARARSVSPKL

SEQ ID NO: 6 - protein, 8 aa, Artificial Sequence
  NSP epitope
RPDTRYVL

SEQ ID NO: 7 - protein, 9 aa, Artificial Sequence
  NSP epitope
TPKYKFVRI

SEQ ID NO: 8 - protein, 9 aa, Artificial Sequence
  NSP epitope
FLLPSLATV

SEQ ID NO: 9 - protein, 9 aa, Artificial Sequence
  NSP epitope
KLWAQCVQL

SEQ ID NO: 10 - protein, 10 aa, Artificial Sequence
  NSP epitope
TEAFEKMVSL

SEQ ID NO: 11 - protein, 9 aa, Artificial Sequence
  NSP epitope
ALWEIQQVV

SEQ ID NO: 12 - protein, 10 aa, Artificial Sequence
  NSP epitope
CTDDNALAYY

SEQ ID NO: 13 - protein, 9 aa, Artificial Sequence
  NSP epitope
VTDTPKGPK

SEQ ID NO: 14 - protein, 10 aa, Artificial Sequence
  NSP epitope
TEVPANSTVL

SEQ ID NO: 15 - protein, 9 aa, Artificial Sequence
  NSP epitope
DLKGKYVQI

SEQ ID NO: 16 - protein, 9 aa, Artificial Sequence
  NSP epitope
LSFKELLVY

SEQ ID NO: 17 - protein, 9 aa, Artificial Sequence
  NSP epitope
IPRRNVATL

SEQ ID NO: 18 - protein, 9 aa, Artificial Sequence
  NSP epitope
MMISAGFSL

SEQ ID NO: 19 - protein, 18 aa, Artificial Sequence
  Accessory protein epitope
TYEGNSPFHPLADNKFAL

SEQ ID NO: 20 - protein, 9 aa, Artificial Sequence
  Accessory protein epitope
RARSVSPKL

SEQ ID NO: 21 - protein, 9 aa, Artificial Sequence
  S epitope
MFIFLLFLT

SEQ ID NO: 22 - protein, 11 aa, Artificial Sequence
  S epitope
KGIYQTSNFRV

SEQ ID NO: 23 - protein, 44 aa, Artificial Sequence
  S epitope
VRFPNITNLCPFGEVFNATRFASVYAWNRKRSNCVADYSVLYNS

SEQ ID NO: 24 - protein, 10 aa, Artificial Sequence
  S epitope
VRQIAPGQTG

SEQ ID NO: 25 - protein, 12 aa, Artificial Sequence
  S epitope
IADYNYKLPDDF

SEQ ID NO: 26 - protein, 15 aa, Artificial Sequence
  S epitope
GYQPYRVVVLSFELL

SEQ ID NO: 27 - protein, 16 aa, Artificial Sequence
  S epitope
CVNFNFNGLTGTGVLT

SEQ ID NO: 28 - protein, 17 aa, Artificial Sequence
  S epitope
NLLLQYGSFCTQLNRAL

SEQ ID NO: 29 - protein, 18 aa, Artificial Sequence
  S epitope
SFIEDLLFNKVTLADAGF

SEQ ID NO: 30 - protein, 20 aa, Artificial Sequence
  S epitope
ARDLICAQKFNGLTVLPPLL

SEQ ID NO: 31 - protein, 37 aa, Artificial Sequence
  S epitope
GWTFGAGAALQIPFAMQMAYRFNGIGVTQNVLYENQK

SEQ ID NO: 32 - protein, 108 aa, Artificial Sequence
  S epitope
ALGKLQDVVNQNAQALNTLVKQLSSNFGAISSVLNDILSRLDKVEAEVQIDRLITGRLQSLQTYVTQQLIRAAEIRASANLAATKMSECVLGQSKRVDFCGKGYHLMS

SEQ ID NO: 33 - protein, 13 aa, Artificial Sequence
  S epitope
APHGVVFLHVTYV

SEQ ID NO: 34 - protein, 20 aa, Artificial Sequence
  S epitope
QIITTDNTFVSGNCDVVIGI

SEQ ID NO: 35 - protein, 82 aa, Artificial Sequence
  S epitope
NTVYDPLQPELDSFKEELDKYFKNHTSPDVDLGDISGINASVVNIQKEIDRLNEVAKNLNESLIDLQELGKYEQYIKWPWYI

SEQ ID NO: 36 - protein, 16 aa, Artificial Sequence
  S epitope
WLGFIAGLIAIVMVTI

SEQ ID NO: 37 - protein, 20 aa, Artificial Sequence
  S epitope
CCKFDEDDSEPVLKGVKLHY

SEQ ID NO: 38 - protein, 53 aa, Artificial Sequence
  E epitope
MYSFVSEETGTLIVNSVLLFLAFVVFLLVTLAILTALRLCAYCCNIVNVSLVK

SEQ ID NO: 39 - protein, 9 aa, Artificial Sequence
  E epitope
YVYSRVKNL

SEQ ID NO: 40 - protein, 11 aa, Artificial Sequence
  M epitope
NRNRFLYIIKL

SEQ ID NO: 41 - protein, 23 aa, Artificial Sequence
  M epitope
FLWLLWPVTLACFVLAAVYRINW

SEQ ID NO: 42 - protein, 27 aa, Artificial Sequence
  M epitope
ASFRLFARTRSMWSFNPETNILLNVPL

SEQ ID NO: 43 - protein, 10 aa, Artificial Sequence
  M epitope
ESELVIGAVI

SEQ ID NO: 44 - protein, 34 aa, Artificial Sequence
  M epitope
GRCDIKDLPKEITVATSRTLSYYKLGASQRVAGD

SEQ ID NO: 45 - protein, 11 aa, Artificial Sequence
  M epitope
RYRIGNYKLNT

SEQ ID NO: 46 - protein, 25 aa, Artificial Sequence
  N epitope
KQRRPQGLPNNTASWFTALTQHGKE

SEQ ID NO: 47 - protein, 10 aa, Artificial Sequence
  N epitope
FPRGQGVPIN

SEQ ID NO: 48 - protein, 16 aa, Artificial Sequence
  N epitope
LSPRWYFYYLGTGPEA

SEQ ID NO: 49 - protein, 34 aa, Artificial Sequence
  N epitope
VLQLPQGTTLPKGFYAEGSRGGSQASSRSSSRSR

SEQ ID NO: 50 - protein, 16 aa, Artificial Sequence
  N epitope
ALALLLLDRLNQLESK

SEQ ID NO: 51 - protein, 30 aa, Artificial Sequence
  N epitope
KGQQQQGQTVTKKSAAEASKKPRQKRTATK

SEQ ID NO: 52 - protein, 19 aa, Artificial Sequence
  N epitope
YNVTQAFGRRGPEQTQGNF

SEQ ID NO: 53 - protein, 43 aa, Artificial Sequence
  N epitope
LIRQGTDYKHWPQIAQFAPSASAFFGMSRIGMEVTPSGTWLTY

SEQ ID NO: 54 - protein, 30 aa, Artificial Sequence
  N epitope
VILLNKHIDAYKTFPPTEPKKDKKKKADET

SEQ ID NO: 55 - protein, 7 aa, Artificial Sequence
  Furin cleavage sites
RGRKRRS

SEQ ID NO: 56 - protein, 18 aa, Artificial Sequence
  leader sequence
MDWTWILFLVAAATRVHS

SEQ ID NO: 57 - protein, 143 aa, Artificial Sequence; identical to SEQ ID NO: 4
  NSP epitope polypeptide sequence

SEQ ID NO: 58 - protein, 474 aa, Artificial Sequence
  S protein epitope polypeptide sequence
MFIFLLFLTAAKGIYQTSNFRVAAVRFPNITNLCPFGEVFNATRFASVYAWNRKRSNCVADYSVLYNSAAGYQPYRVVVLSFELLAACVNFNFNGLTGTGVLTAANLLLQYGSFCTQLNRALAASFIEDLLFNKVTLADAGFAAARDLICAQKFNGLTVLPPLLAAGWTFGAGAALQIPFAMQMAYRFNGIGVTQNVLYENQKAAALGKLQDVVNQNAQALNTLVKQLSSNFGAISSVLNDILSRLDKVEAEVQIDRLITGRLQSLQTYVTQQLIRAAEIRASANLAATKMSECVLGQSKRVDFCGKGYHLMSAAAPHGVVFLHVTYVAAQIITTDNTFVSGNCDVVIGIAANTVYDPLQPELDSFKEELDKYFKNHTSPDVDLGDISGINASVVNIQKEIDRLNEVAKNLNESLIDLQELGKYEQYIKWPWYIAAWLGFIAGLIAIVMVTIAACCKFDEDDSEPVLKGVKLHY

SEQ ID NO: 59 - protein, 126 aa, Artificial Sequence
  M protein epitope polypeptide sequence
NRNRFLYIIKLAAFLWLLWPVTLACFVLAAVYRINWAAASFRLFARTRSMWSFNPETNILLNVPLAAESELVIGAVIAAGRCDIKDLPKEITVATSRTLSYYKLGASQRVAGDAARYRIGNYKLNT

SEQ ID NO: 60 - protein, 239 aa, Artificial Sequence
  N protein epitope polypeptide sequence
KQRRPQGLPNNTASWFTALTQHGKEAAFPRGQGVPINAALSPRWYFYYLGTGPEAAAVLQLPQGTTLPKGFYAEGSRGGSQASSRSSSRSRAAALALLLLDRLNQLESKAAKGQQQQGQTVTKKSAAEASKKPRQKRTATKAAYNVTQAFGRRGPEQTQGNFAALIRQGTDYKHWPQIAQFAPSASAFFGMSRIGMEVTPSGTWLTYAAVILLNKHIDAYKTFPPTEPKKDKKKKADET